European Patent Application EP 4 541 900 A2, published April 23, 2025. Title: COMPOSITION AND METHODS OF GENOME EDITING OF B-CELLS. Applicant: Dana-Farber Cancer Institute, Inc. The sequence listing filed with the application follows.

SEQUENCE LISTING (24 sequences)

SEQ ID NO: 1 - protein, 9 aa, synthetic construct
  REGION 1..9: note = Synthetic Polypeptide
LAGLIDADG

SEQ ID NO: 2 - protein, 6 aa, synthetic construct
  REGION 1..6: note = Synthetic Polypeptide
GIYYIG

SEQ ID NO: 3 - protein, 5 aa, synthetic construct
  REGION 1..5: note = Synthetic Polypeptide
TGEKP

SEQ ID NO: 4 - protein, 6 aa, synthetic construct
  REGION 1..6: note = Synthetic Polypeptide
TGGQRP

SEQ ID NO: 5 - protein, 5 aa, synthetic construct
  REGION 1..5: note = Synthetic Polypeptide
TGQKP

SEQ ID NO: 6 - protein, 6 aa, synthetic construct
  REGION 1..6: note = Synthetic Polypeptide
TGSQKP

SEQ ID NO: 7 - DNA, 20 bp, synthetic construct
  misc_feature 1..20: note = Synthetic Polynucleotide
  source 1..20: mol_type = other DNA
gaaaacacctgaaaatccca

SEQ ID NO: 8 - DNA, 20 bp, synthetic construct
  misc_feature 1..20: note = Synthetic Polynucleotide
  source 1..20: mol_type = other DNA
gtcctcggggcatgttccga

SEQ ID NO: 9 - DNA, 20 bp, synthetic construct
  misc_feature 1..20: note = Synthetic Polynucleotide
  source 1..20: mol_type = other DNA
ttaggacccagagggaacca

SEQ ID NO: 10 - DNA, 20 bp, synthetic construct
  misc_feature 1..20: note = Synthetic Polynucleotide
  source 1..20: mol_type = other DNA
ctgtggctcactttcggcgg

SEQ ID NO: 11 - DNA, 20 bp, synthetic construct
  misc_feature 1..20: note = Synthetic Polynucleotide
  source 1..20: mol_type = other DNA
tgaacagagagaactcacca

SEQ ID NO: 12 - DNA, 20 bp, synthetic construct
  misc_feature 1..20: note = Synthetic Polynucleotide
  source 1..20: mol_type = other DNA
ggtcctcggggcatgttccg

SEQ ID NO: 13 - DNA, 20 bp, synthetic construct
  misc_feature 1..20: note = Synthetic Polynucleotide
  source 1..20: mol_type = other DNA
gctgctcagttaggacccag

SEQ ID NO: 14 - DNA, 20 bp, synthetic construct
  misc_feature 1..20: note = Synthetic Polynucleotide
  source 1..20: mol_type = other DNA
gggcatttaagatttgccat

SEQ ID NO: 15 - DNA, 1413 bp, synthetic construct
  misc_feature 1..1413: note = Synthetic Polynucleotide
  source 1..1413: mol_type = other DNA
atggagttcggcctgagctggctgttcctggtggccatcctgaagggcgtgcagtgcgaggtgcagctggtggagagcggcggcggcctggtgcagcccggcagaagcctgagactgagctgcgccgccagcggcttcaccttcgacgactacgccatgcactgggtgagacaggcccccggcaagggcctggagtgggtgagcgccatcacctggaacagcggccacatcgactacgccgacagcgtggagggcagattcaccatcagcagagacaacgccaagaacagcctgtacctgcagatgaacagcctgagagccgaggacaccgccgtgtactactgcgccaaggtgagctacctgagcaccgccagcagcctggactactggggccagggcaccctggtgaccgtgagcagcgccagcaccaagggccccagcgtgttccccctggcccccagcagcaagagcaccagcggcggcaccgccgccctgggctgcctggtgaaggactacttccccgagcccgtgaccgtgagctggaacagcggcgccctgaccagcggcgtgcacaccttccccgccgtgctgcagagcagcggcctgtacagcctgagcagcgtggtgaccgtgcccagcagcagcctgggcacccagacctacatctgcaacgtgaaccacaagcccagcaacaccaaggtggacaagaaggtggagcccaagagctgcgacaagacccacacctgccccccctgccccgcccccgagctgctgggcggccccagcgtgttcctgttcccccccaagcccaaggacaccctgatgatcagcagaacccccgaggtgacctgcgtggtggtggacgtgagccacgaggaccccgaggtgaagttcaactggtacgtggacggcgtggaggtgcacaacgccaagaccaagcccagagaggagcagtacaacagcacctacagagtggtgagcgtgctgaccgtgctgcaccaggactggctgaacggcaaggagtacaagtgcaaggtgagcaacaaggccctgcccgcccccatcgagaagaccatcagcaaggccaagggccagcccagagagccccaggtgtacaccctgccccccagcagagacgagctgaccaagaaccaggtgagcctgacctgcctggtgaagggcttctaccccagcgacatcgccgtggagtgggagagcaacggccagcccgagaacaactacaagaccaccccccccgtgctggacagcgacggcagcttcttcctgtacagcaagctgaccgtggacaagagcagatggcagcagggcaacgtgttcagctgcagcgtgatgcacgaggccctgcacaaccactacacccagaagagcctgagcctgagccccggcaagtga

SEQ ID NO: 16 - DNA, 711 bp, synthetic construct
  misc_feature 1..711: note = Synthetic Polynucleotide
  source 1..711: mol_type = other DNA
atggacatgagagtgcccgcccagctgctgggcctgctgctgctgtggctgcccgacaccagatgcgacatccagatgacccagagccccagcagcctgagcgccagcgtgggcgacagagtgaccatcacctgcagagccagccagggcatcagaaactacctggcctggtaccagcagaagcccggcaaggcccccaagctgctgatctacgccgccagcaccctgcagagcggcgtgcccagcagattcagcggcagcggcagcggcaccgacttcaccctgaccatcagcagcctgcagcccgaggacgtggccacctactactgccagagatacaacagagccccctacaccttcggccagggcaccaaggtggagatcaagagaaccgtggccgcccccagcgtgttcatcttcccccccagcgacgagcagctgaagagcggcaccgccagcgtggtgtgcctgctgaacaacttctaccccagagaggccaaggtgcagtggaaggtggacaacgccctgcagagcggcaacagccaggagagcgtgaccgagcaggacagcaaggacagcacctacagcctgagcagcaccctgaccctgagcaaggccgactacgagaagcacaaggtgtacgcctgcgaggtgacccaccagggcctgagcagccccgtgaccaagagcttcaacagaggcgagtgctga

SEQ ID NO: 17 - DNA, 201 bp, synthetic construct
  misc_feature 1..201: note = Synthetic Polynucleotide
  source 1..201: mol_type = other DNA
tatatagtaggagatatgcaaatagagccctccgtctgctgatgaaaaccagcccagccctgaccctgcagctctgagagaggagcccagaagcttggatcccaggtgttttcatttggtgatcaggactgaacagagagaactcaccatggagtttgggctgagctggctttttctttgtggctattttaaaaggtaatt

SEQ ID NO: 18 - DNA, 199 bp, synthetic construct
  misc_feature 1..199: note = Synthetic Polynucleotide
  source 1..199: mol_type = other DNA
agtaggagatatgcaaatagagccctccgtctgctgatgaaaaccagcccagccctgaccctgcagctctgagagaggagccagatggactacaaagacgatgacgacaagtgaatttggtgatcaggactgaacagagagaactcaccatggagtttgggctgagctggctttttcttgtggctattttaaaaggtaa

SEQ ID NO: 19 - DNA, 200 bp, synthetic construct
  misc_feature 1..200: note = Synthetic Polynucleotide
  source 1..200: mol_type = other DNA
tatatagtaggagatatgcaaatagagccctccgtctgctgatgaaaaccagcccagccctgaccctgcagctctgagagaggagcccagaagcttggatcccaggtgttttcggacctgggcggactggccaggaggggatgggcactggggtgccttgaggatctgggagcctctgtggattttccgatgcctttgga

SEQ ID NO: 20 - DNA, 200 bp, synthetic construct
  misc_feature 1..200: note = Synthetic Polynucleotide
  source 1..200: mol_type = other DNA
agtaggagatatgcaaatagagccctccgtctgctgatgaaaaccagcccagccctgaccctgcagctctgagagaggagcccagatggactacaaagacgatgacgacaagtgaggacctgggcggactggccaggaggggatgggcactggggtgccttgaggatctgggagcctctgtggattttccgatgcctttg

SEQ ID NO: 21 - DNA, 200 bp, synthetic construct
  misc_feature 1..200: note = Synthetic Polynucleotide
  source 1..200: mol_type = other DNA
cccagctgctttgcatgtccctcccagccgccctgcagtccagagcccatatcaatgcctgggtcagagctctggagaagagctgctcagttaggacccagaagcttggatccaaaccccagcgcagcttctcttcctcctgctactctggctcccaggtgaggggaacatgggatggttttgcatgtcagtgaaaaccc

SEQ ID NO: 22 - DNA, 200 bp, synthetic construct
  misc_feature 1..200: note = Synthetic Polynucleotide
  source 1..200: mol_type = other DNA
ctgctttgcatgtccctcccagccgccctgcagtccagagcccatatcaatgcctgggtcagagctctggagaagagctgctcagatgtacccatacgatgttccagattacgcttgaaaaccccagcgcagcttctcttcctcctgctactctggctcccaggtgaggggaacatgggatggttttgcatgtcagtgaa

SEQ ID NO: 23 - DNA, 201 bp, synthetic construct
  misc_feature 1..201: note = Synthetic Polynucleotide
  source 1..201: mol_type = other DNA
cccagctgctttgcatgtccctcccagccgccctgcagtccaagagcccatatcaatgcctgggtcagagctctggagaagagctgctcagttaggacccagaagcttggatccgaccaaggtggagatcaaacgtaagtgcactttcctaatgctttttcttataaggttttaaatttggagcgtttttgtgtttgagat

SEQ ID NO: 24 - DNA, 200 bp, synthetic construct
  misc_feature 1..200: note = Synthetic Polynucleotide
  source 1..200: mol_type = other DNA
ctgctttgcatgtccctcccagccgccctgcagtccagagcccatatcaatgcctgggtcagagctctggagaagagctgctcagatgtacccatacgatgttccagattacgcttgagaccaaggtggagatcaaacgtaagtgcactttcctaatgctttttcttataaggttttaaatttggagcgtttttgtgttt